European Patent Application EP 4 257 683 A1, published October 11, 2023. Title: Neue Urethanasen für den enzymatischen Abbau von Polyurethanen. Applicant: Covestro Deutschland AG. The sequence listing filed with the application follows.

SEQUENCE LISTING (1 sequence)

SEQ ID NO: 1 - protein, 440 aa, Derived from metagenome
MAREPTALATAAAIRSGATTARAETEAAIARIEALDGAINAVVVRDFDRALAAADAADARIQAGDTAPLLGVPMTVKEAFDVEGLPTHWGFRQHAGNIATSDAEAVRRLKAAGAIILGKTNVPKGLGDWQSVNSIHGVTNHPLDPTRTPGGSSGGSAAALASGMVPLELGSDIGGSIRIPAHFCGVWGLKPSWGAISSHGHRYPGTNGAETPLGVIGPMARSPDDLAAMLDLLATLPMPRASRPPRRVLAITDHPAIRTSAVCRDAVDTAAEALAGAGIEVIRSTDLLPDLARQHHAYGQMLSVAFARSDPTLHASLPNLLTWLSWQDAQARNTRAWGRLFGEVDAVIAPPAATQAFAHDHAPQANRTLDIDGVASPYDAHLAWAGVATYPGLPAVVVPVGTANGLPVGVQVITDFHRDHDAIATAALIHRLTEGQPALE